European Patent Specification EP 4 025 915 B1, published November 26, 2025. Title: Assay for assessing Heart failure. Applicant: Nordic Bioscience A/S. The sequence listing filed with the application follows.

SEQUENCE LISTING (8 sequences)

SEQ ID NO: 1 - protein, 7 aa, Artificial Sequence
  C-terminus sequence
QETCIQG

SEQ ID NO: 2 - protein, 8 aa, Artificial Sequence
  elongated sequence
QETCIQGA

SEQ ID NO: 3 - protein, 6 aa, Artificial Sequence
  truncated sequence
QETCIQ

SEQ ID NO: 4 - protein, 7 aa, Artificial Sequence
  SITE 1: biotinylated at N-terminus with optional linker
  biotinylated peptide
QETCIQG

SEQ ID NO: 5 - protein, 10 aa, Artificial Sequence
  C-terminus sequence
KECQETCIQG

SEQ ID NO: 6 - protein, 10 aa, Artificial Sequence
  SITE 1: KLH attatched to N-terminus
  immunogenic peptide
CGGQETCIQG

SEQ ID NO: 7 - protein, 10 aa, Artificial Sequence
  non-sense peptide
GLRPGSEYTV

SEQ ID NO: 8 - protein, 11 aa, Artificial Sequence
  non-sesnse coater
  SITE 11: biotinylated at C-terminus
GLRPGSEYTVK